European Patent Specification EP 3 584 316 B1, published April 3, 2024. Title: Bacterial delivery vehicle, process of production and uses thereof. Applicant: Eligo Bioscience. The sequence listing filed with the application follows.

SEQUENCE LISTING (6 sequences)

SEQ ID NO: 1 - DNA, 791 bp, artificial
  P1 Pac
acctgggacgatcacaagaagaattttgctcgcctggcgcgagatggtggttacaccatcgcacagtatgccgccgagtttaatcttaaccctaataccgcacgtcgttatctccgtgccttcaaagaggacaccaggactacggacagccgcaagccaaataagccagtcaggaagccactaaaaagcatgatcattgatcactctaatgatcaacatgcaggtgatcacattgcggctgaaatagcggaaaaacaaagagttaatgccgttgtcagtgccgcagtcgagaatgcgaagcgccaaaataagcgcataaatgatcgttcagatgatcatgacgtgatcacccgcgcccaccggaccttacgtgatcgcctggaacgcgacaccctggatgatgatggtgaacgctttgagttcgaagttggcgattacctgatagataacgttgaagcgcggaaggccgcgcgcgctatgttgcgtcggtccggggccgatgttctggaaaccactcttctggaaaagtctctttctcatctccttatgctggagaacgccagggatacgtgtattcgcctggtgcaggaaatgcgcgatcagcaaaaagacgatgatgaaggtactccgcctgaataccgtatcgcgagcatgctaaacagctgttccgcgcagataagcagcctgatcaacaccatttacagcatccggaataactatcgaaaagaaagccgggaggcggaaaagcacgctttatctatggggcaagctggcattgttaagctggcata

SEQ ID NO: 2 - DNA, 325 bp, artificial
  Cos P4
gcatgcgttttcctgcctcattttctgcaaaccgcgccattcccggcgcggtctgagcgtgtcagtgcaactgcattaaaaccgccccgcaaagcgggcgggcgaggcggggaaagcaccgcgcgcaaaccgacaagttagttaattatttgtgtagtcaaagtgccttcagtacatacctcgttaatacattggagcataatgaagaaaatctatggcctatggtccaaaactgtcttttttgatggcactatcctgaaaaatatgcaaaaaatagattgatgtaaggtggttcttgtcagtgtcgcaagatccttaagaattc

SEQ ID NO: 3 - DNA, 224 bp, artificial
  Cos lambda
ccaaaaagcctcgctttcagcacctgtcgtttcctttcttttcagagggtattttaaataaaaacattaagttatgacgaagaagaacggaaacgccttaaaccggaaaattttcataaatagcgaaaacccgcgaggtcgccgccccgtaacctgtcggatcaccggaaaggacccgtaaagtgataatgattatcatctacatatcacaacgtgcgtaaagg

SEQ ID NO: 4 - DNA, 84 bp, artificial
  Cos P2
taaggtgcattaaaaccgccccgtgaagcgggcgggcgaggcggggaaagcacggcgaggcggggaaagcactgcgcgctgacg

SEQ ID NO: 5 - DNA, 140 bp, artificial
  Cos 186
tgttttgcatgcgtcaggcttgcccgttctggttgtgcgtcgccagagctggcgcggctccagagtggtcatgcaactgcattaaaaccgacccataaagtgggcaggcgtggcggggaaagcattgcgcgccagaggtg

SEQ ID NO: 6 - DNA, 1115 bp, artificial
  T7 concatemer junction
agtccatgcagttggattccgttaaggtcgagggtgaagtacttgctgacttccttgaggaacacatgatgcgtcctacggttgctgctacgcatatcattgagatgtctgtgggaggagttgatgtgtactctgaggacgatgagggttacggtacgtctttcattgagtggtgatttatgcattaggactgcatagggatgcactatagaccacggatggtcagttctttaagttactgaaaagacacgataaattaatacgactcactatagggagaggagggacgaaaggttactatatagatactgaatgaatacttatagagtgcataaagtatgcataatggtgtacctagagtgacctctaagaatggtgattatattgtattagtatcaccttaacttaaggaccaacataaagggaggagactcatgttccgcttattgttgaacctactgcggcatagagtcacctaccgatttcttgtggtactttgtgctgcccttgggtacgcatctcttactggagacctcagttcactggagtctgtcgtttgctctatactcacttgtagcgattagggtcttcctgaccgactgatggctcaccgagggattcagcggtatgattgcatcacaccacttcatccctatagagtcaagtcctaaggtatacccataaagagcctctaatggtctatcctaaggtctatacctaaagataggccatcctatcagtgtcacctaaagagggtcttagagagggcctatggagttcctatagggtcctttaaaatataccataaaaatctgagtgactatctcacagtgtacggacctaaagttcccccatagggggtacctaaagcccagccaatcacctaaagtcaaccttcggttgaccttgagggttccctaagggttggggatgacccttgggtttgtctttgggtgttaccttgagtgtctctctgtgtccctatctgttacagtctcctaaagtatcctcctaaagtcacctcctaacgtccatcctaaagccaacacctaaagcctacacctaaagacccatcaagtcaacgcctatcttaaagtttaaacataaagaccaga